European Patent Application EP 4 491 731 A1, published January 15, 2025. Title: Modified Proteinglutaminase. Applicant: Amano Enzyme Inc. The sequence listing filed with the application follows.

SEQUENCE LISTING (23 sequences)

SEQ ID NO: 1 - protein, 185 aa, Chryseobacterium proteolyticum
LASVIPDVATLNSLFNQIKNQSCGTSTASSPCITFRYPVDGCYARAHKMRQILMNNGYDCEKQFVYGNLKASTGTCCVAWSYHVAILVSYKNASGVTEKRIIDPSLFSSGPVTDTAWRNACVNTSCGSASVSSYANTAGNVYYRSPSNSYLYDNNLINTNCVLTKFSLLSGCSPSPAPDVSSCGF

SEQ ID NO: 2 - protein, 11 aa, synthetic construct
  REGION 1..11: note = A sequence newly found to impart the property of inhibiting thedecrease in reactivity at high temperature to proteinglutaminaseby the present invention.
RYGVKMSNQDG

SEQ ID NO: 3 - protein, 320 aa, Chryseobacterium proteolyticum
MKNLFLSMMAFVTVLTFNSCADSNGNQEINGKEKLSVNDSKLKDFGKTVPVGIDEENGMIKVSFMLTAQFYEIKPTKENEQYIGMLRQAVKNESPVHIFLKPNSNEIGKVESASPEDVRYFKTILTKEVKGQTNKLASVIPDVATLNSLFNQIKNQSCGTSTASSPCITFRYPVDGCYARAHKMRQILMNNGYDCEKQFVYGNLKASTGTCCVAWSYHVAILVSYKNASGVTEKRIIDPSLFSSGPVTDTAWRNACVNTSCGSASVSSYANTAGNVYYRSPSNSYLYDNNLINTNCVLTKFSLLSGCSPSPAPDVSSCGF

SEQ ID NO: 4 - protein, 185 aa, synthetic construct
  REGION 1..185: note = P38A mutation of proteinglutaminase derived from Chryseobacteriumproteolyticum
LASVIPDVATLNSLFNQIKNQSCGTSTASSPCITFRYAVDGCYARAHKMRQILMNNGYDCEKQFVYGNLKASTGTCCVAWSYHVAILVSYKNASGVTEKRIIDPSLFSSGPVTDTAWRNACVNTSCGSASVSSYANTAGNVYYRSPSNSYLYDNNLINTNCVLTKFSLLSGCSPSPAPDVSSCGF

SEQ ID NO: 5 - protein, 185 aa, synthetic construct
  REGION 1..185: note = L156Y mutation of proteinglutaminase derived fromChryseobacterium proteolyticum
LASVIPDVATLNSLFNQIKNQSCGTSTASSPCITFRYPVDGCYARAHKMRQILMNNGYDCEKQFVYGNLKASTGTCCVAWSYHVAILVSYKNASGVTEKRIIDPSLFSSGPVTDTAWRNACVNTSCGSASVSSYANTAGNVYYRSPSNSYLYDNNYINTNCVLTKFSLLSGCSPSPAPDVSSCGF

SEQ ID NO: 6 - protein, 192 aa, synthetic construct
  REGION 1..192: note = S72-T75 to RYGVKMSNQDG mutation of proteinglutaminase derivedfrom Chryseobacterium proteolyticum
LASVIPDVATLNSLFNQIKNQSCGTSTASSPCITFRYPVDGCYARAHKMRQILMNNGYDCEKQFVYGNLKARYGVKMSNQDGCCVAWSYHVAILVSYKNASGVTEKRIIDPSLFSSGPVTDTAWRNACVNTSCGSASVSSYANTAGNVYYRSPSNSYLYDNNLINTNCVLTKFSLLSGCSPSPAPDVSSCGF

SEQ ID NO: 7 - protein, 185 aa, Chryseobacterium sp.
AVSVIPNLATLNSLFTQIKNQACGTSTASSPCITFRYPVDGCYARAHKMRQILLNAGYDCEKQFVYGNLRASTGTCCVSWVYHVAILVSFKNASGIVEKRIIDPSLFSSGPVTDAAWRAACTNTSCGSASVSSYANTAGNVYYRSPSGSLLYDNNYVNTNCVLNIFSSLSGCSPSPAPSVASCGF

SEQ ID NO: 8 - protein, 185 aa, Chryseobacterium sp.
AVSVIPNLATLNSLFTQIKNQACGTSTASSPCITFRYPVDGCYARAHKMRQILLNAGYDCEKQFVYGNLRASTGTCCVSWVYHVAILVSFKNASGIVEKRIIDPSLFSSGPVTDTAWRAACTNTSCGSASVSSYANTAGNVYYRSPSGSLLYDNNYVNTNCVLNIFSSLSGCSPSPAPSVASCGF

SEQ ID NO: 9 - protein, 319 aa, Chryseobacterium sp.
MKKFLLSMMVFVTMLSFNACSDSAANQDPNLVAKESNEIAMKDFGKTVPVGIEKEEGKFKVSFMVSAQPYHIKDSKENAGYISMIRQAVENETPVHIFLKTNTTEIAKVDKPTDDDIRYFKSVFNKEERGDSKKAVSVIPNLATLNSLFTQIKNQACGTSTASSPCITFRYPVDGCYARAHKMRQILLNAGYDCEKQFVYGNLRASTGTCCVSWVYHVAILVSFKNASGIVEKRIIDPSLFSSGPVTDAAWRAACTNTSCGSASVSSYANTAGNVYYRSPSGSLLYDNNYVNTNCVLNIFSSLSGCSPSPAPSVASCGF

SEQ ID NO: 10 - protein, 319 aa, Chryseobacterium sp.
MKKFLLSMMVFVTVLSFNSCSDSSANQDPNLVAKESNEIAMKDFGKTVPVGIEKEDGKFKVSFIVSAQPYQIKDTKENAGYISMIKEAVENETPVQVFLKANSNEIAKVDKATADDIRYFKSVFNKEERGDSRKAVSVIPNLATLNSLFTQIKNQACGTSTASSPCITFRYPVDGCYARAHKMRQILLNAGYDCEKQFVYGNLRASTGTCCVSWVYHVAILVSFKNASGIVEKRIIDPSLFSSGPVTDTAWRAACTNTSCGSASVSSYANTAGNVYYRSPSGSLLYDNNYVNTNCVLNIFSSLSGCSPSPAPSVASCGF

SEQ ID NO: 11 - DNA, 558 bp, Chryseobacterium proteolyticum
  source 1..558: mol_type = other DNA
ttggcgagtgtaattcctgatgtagctacattaaattctttattcaatcaaataaagaatcagtcttgcggtacctctacggcgtcctcaccatgcatcacattcagatatcctgtagacggatgttatgcaagagcccataagatgagacaaatcttaatgaacaacggctatgactgtgaaaaacaatttgtatacggaaacctaaaggcatcaacaggaacttgctgtgtggcgtggagctaccacgttgcaatattggtaagctataaaaatgcttccggagtaacggaaaaaagaattattgatccttcactattttcaagcggtcctgtaacagatacagcatggagaaacgcttgcgttaacacctcttgcggatctgcatccgtttcctcttatgctaatactgcaggaaatgtttattacagaagtcctagtaattcttacctgtatgacaacaatctgatcaataccaactgtgtactgactaaattttcactgctttccggatgttctccttcacctgcaccggatgtatccagctgtggattttaa

SEQ ID NO: 12 - DNA, 558 bp, synthetic construct
  misc_feature 1..558: note = DNA coding P38A mutation of proteinglutaminase derived fromChryseobacterium proteolyticum
  source 1..558: mol_type = other DNA
ttggcgagtgtaattcctgatgtagctacattaaattctttattcaatcaaataaagaatcagtcttgcggtacctctacggcgtcctcaccatgcatcacattcagatatgctgtagacggatgttatgcaagagcccataagatgagacaaatcttaatgaacaacggctatgactgtgaaaaacaatttgtatacggaaacctaaaggcatcaacaggaacttgctgtgtggcgtggagctaccacgttgcaatattggtaagctataaaaatgcttccggagtaacggaaaaaagaattattgatccttcactattttcaagcggtcctgtaacagatacagcatggagaaacgcttgcgttaacacctcttgcggatctgcatccgtttcctcttatgctaatactgcaggaaatgtttattacagaagtcctagtaattcttacctgtatgacaacaatctgatcaataccaactgtgtactgactaaattttcactgctttccggatgttctccttcacctgcaccggatgtatccagctgtggattttaa

SEQ ID NO: 13 - DNA, 558 bp, synthetic construct
  misc_feature 1..558: note = DNA coding L156Y mutation of proteinglutaminase derived fromChryseobacterium proteolyticum
  source 1..558: mol_type = other DNA
ttggcgagtgtaattcctgatgtagctacattaaattctttattcaatcaaataaagaatcagtcttgcggtacctctacggcgtcctcaccatgcatcacattcagatatcctgtagacggatgttatgcaagagcccataagatgagacaaatcttaatgaacaacggctatgactgtgaaaaacaatttgtatacggaaacctaaaggcatcaacaggaacttgctgtgtggcgtggagctaccacgttgcaatattggtaagctataaaaatgcttccggagtaacggaaaaaagaattattgatccttcactattttcaagcggtcctgtaacagatacagcatggagaaacgcttgcgttaacacctcttgcggatctgcatccgtttcctcttatgctaatactgcaggaaatgtttattacagaagtcctagtaattcttacctgtatgacaacaattacatcaataccaactgtgtactgactaaattttcactgctttccggatgttctccttcacctgcaccggatgtatccagctgtggattttaa

SEQ ID NO: 14 - DNA, 579 bp, synthetic construct
  misc_feature 1..579: note = DNA coding S72-T75 to RYGVKMSNQDG mutation of proteinglutaminasederived from Chryseobacterium proteolyticum
  source 1..579: mol_type = other DNA
ttggcgagtgtaattcctgatgtagctacattaaattctttattcaatcaaataaagaatcagtcttgcggtacctctacggcgtcctcaccatgcatcacattcagatatcctgtagacggatgttatgcaagagcccataagatgagacaaatcttaatgaacaacggctatgactgtgaaaaacaatttgtatacggaaacctaaaggcacgttatggcgttaagatgtcaaaccaggatggttgctgtgtggcgtggagctaccacgttgcaatattggtaagctataaaaatgcttccggagtaacggaaaaaagaattattgatccttcactattttcaagcggtcctgtaacagatacagcatggagaaacgcttgcgttaacacctcttgcggatctgcatccgtttcctcttatgctaatactgcaggaaatgtttattacagaagtcctagtaattcttacctgtatgacaacaatctgatcaataccaactgtgtactgactaaattttcactgctttccggatgttctccttcacctgcaccggatgtatccagctgtggattttaa

SEQ ID NO: 15 - DNA, 963 bp, Chryseobacterium proteolyticum
  source 1..963: mol_type = other DNA
atgaaaaatctttttttatcaatgatggcctttgtgaccgtcttaacttttaattcctgtgccgattccaacgggaatcaggaaatcaacggaaaggaaaaactaagtgtaaatgattctaagctgaaagatttcggaaagactgtaccggtagggatagacgaagaaaacggaatgataaaggtgtcatttatgttaactgcgcaattctatgaaattaagccgaccaaagaaaatgagcagtatatcggaatgcttagacaggctgttaagaatgaatctcctgtacacattttcttaaagcctaatagcaatgaaataggaaaagtggagtctgcaagtccggaagacgtaagatattttaaaacgatcctgacaaaagaagtaaaagggcaaaccaataaattggcgagtgtaattcctgatgtagctacattaaattctttattcaatcaaataaagaatcagtcttgcggtacctctacggcgtcctcaccatgcatcacattcagatatcctgtagacggatgttatgcaagagcccataagatgagacaaatcttaatgaacaacggctatgactgtgaaaaacaatttgtatacggaaacctaaaggcatcaacaggaacttgctgtgtggcgtggagctaccacgttgcaatattggtaagctataaaaatgcttccggagtaacggaaaaaagaattattgatccttcactattttcaagcggtcctgtaacagatacagcatggagaaacgcttgcgttaacacctcttgcggatctgcatccgtttcctcttatgctaatactgcaggaaatgtttattacagaagtcctagtaattcttacctgtatgacaacaatctgatcaataccaactgtgtactgactaaattttcactgctttccggatgttctccttcacctgcaccggatgtatccagctgtggattttaa

SEQ ID NO: 16 - DNA, 960 bp, Chryseobacterium sp.
  source 1..960: mol_type = other DNA
atgaaaaaatttctgttatccatgatggtattcgtgacgatgctgtcattcaatgcctgttcagattcagctgccaatcaggatcccaatcttgttgctaaagagtctaatgaaatcgccatgaaagatttcggtaaaactgttccggtagggattgaaaaagaagagggaaaatttaaagtctcttttatggtgagtgctcagccataccacattaaagacagtaaggaaaatgcaggttatatttctatgatcagacaagccgttgaaaacgaaactcctgttcatattttcctgaaaaccaacaccactgaaattgcaaaagtagataaacctactgatgatgatatccgttatttcaaatctgttttcaataaagaagagagaggagacagcaaaaaagcagtgagtgttattcctaacctggcaacactgaacagcttatttacgcagattaaaaaccaggcttgcggtacttctacagcatcttctccatgtatcactttcagatatccggtggatggatgttatgcaagagctcacaaaatgagacagatcctccttaatgcaggctacgactgtgaaaagcagttcgtttacggaaacctgagagcttctacaggaacttgctgcgtatcatgggtatatcacgtagccatattggtaagcttcaaaaatgcttccggaattgttgagaaaagaatcatcgatccttcactattctccagcggacccgtaactgacgcagcatggagagccgcttgtaccaacacaagctgtggatctgcttctgtatcttcttatgccaatacagcaggaaacgtgtactacagaagtccatcaggatctttactgtatgataacaattatgtaaataccaattgtgtattgaatatattctcatccctttcaggatgttctccttctcctgcaccaagtgtagcgagctgcggattttaa

SEQ ID NO: 17 - DNA, 960 bp, Chryseobacterium sp.
  source 1..960: mol_type = other DNA
atgaaaaaatttcttttatccatgatggtattcgtgacggtactttcatttaactcctgttcggattcaagtgccaatcaggatccgaatcttgttgctaaagagtctaatgaaattgctatgaaagactttggtaaaactgttccggtagggatagaaaaagaggatggaaagtttaaagtttcctttatagtttcagcgcagccgtatcaaattaaagatacaaaagaaaatgcgggatatatctccatgatcaaagaggctgtagaaaatgaaactcctgttcaggttttcctgaaagccaattctaacgaaatcgcaaaggtagacaaagcaacagcggatgacatccgttatttcaaatctgttttcaacaaagaagagagaggcgacagcagaaaagctgtgagcgttattcctaatcttgcaacgctgaacagcttattcactcagatcaaaaaccaggcttgcggaacttctacagcatcttcaccgtgtatcacattcagatatcctgtggatggatgctatgcgagagctcacaaaatgagacaaatccttttgaatgcaggctacgactgtgaaaaacagttcgtttacgggaacctaagagcatctacaggaacatgctgtgtgtcttgggtatatcacgtagccattttggtaagcttcaaaaatgcttccggaattgttgagaaaagaattattgatccgtcactattctccagcggacctgtaacagatactgcatggagagccgcatgtaccaacacaagctgtggatctgcttctgtttcttcttatgccaatacagcaggaaatgtatactacagaagcccatccggttctttattatatgataacaattatgtaaataccaactgtgtattgaacatattctcatccctttcaggatgttctccttcccctgcacctagtgtagcaagctgtggattttaa

SEQ ID NO: 18 - DNA, 27 bp, synthetic construct
  misc_feature 1..27: note = synthetic primer
  source 1..27: mol_type = other DNA
agatatgctgtagacggatgttatgca

SEQ ID NO: 19 - DNA, 27 bp, synthetic construct
  misc_feature 1..27: note = synthetic primer
  source 1..27: mol_type = other DNA
gtctacagcatatctgaatgtgatgca

SEQ ID NO: 20 - DNA, 27 bp, synthetic construct
  misc_feature 1..27: note = synthetic primer
  source 1..27: mol_type = other DNA
aacaattacatcaataccaactgtgta

SEQ ID NO: 21 - DNA, 27 bp, synthetic construct
  misc_feature 1..27: note = synthetic primer
  source 1..27: mol_type = other DNA
attgatgtaattgttgtcatacaggta

SEQ ID NO: 22 - DNA, 42 bp, synthetic construct
  misc_feature 1..42: note = synthetic primer
  source 1..42: mol_type = other DNA
tgtcaaaccaggatggttgctgtgtggcgtggagctaccacg

SEQ ID NO: 23 - DNA, 41 bp, synthetic construct
  misc_feature 1..41: note = synthetic primer
  source 1..41: mol_type = other DNA
tcttaacgccataacgtgcctttaggtttccgtatacaaat